European Patent Application EP 4 413 999 A2, published August 14, 2024. Title: FLT3-SPECIFIC CHIMERIC ANTIGEN RECEPTORS AND METHODS USING SAME. Applicant: THE UNITED STATES OF AMERICA, AS REPRESENTED BY THE SECRETARY, DEPARTMENT OF HEALTH AND HUMAN SERVICES. The sequence listing filed with the application follows.

SEQUENCE LISTING (30 sequences)

SEQ ID NO: 1 - protein, 490 aa, synthetic construct
  REGION 1..490: note = SYNTHETIC
MLLVTSLLLCELPHPAFLLIPEVQLVQSGAEVKKPGSSVKVSCKASGGTFSSYAISWVRQAPGQGLEWMGGIIPIFGTANYAQKFQGRVTITADKSTSTAYMELSSLRSEDTAVYYCATFALFGFREQAFDIWGQGTTVTVSSGGGGSGGGGSGGGGSDIQMTQSPSSLSASVGDRVTITCRASQSISSYLNWYQQKPGKAPKLLIYAASSLQSGVPSRFSGSGSGTDFTLTISSLQPEDLATYYCQQSYSTPFTFGPGTKVDIKSGTTTPAPRPPTPAPTIASQPLSLRPEACRPAAGGAVHTRGLDFACDIYIWAPLAGTCGVLLLSLVITLYCKRGRKKLLYIFKQPFMRPVQTTQEEDGCSCRFPEEEEGGCELRVKFSRSADAPAYKQGQNQLYNELNLGRREEYDVLDKRRGRDPEMGGKPRRKNPQEGLYNELQKDKMAEAYSEIGMKGERRRGKGHDGLYQGLSTATKDTYDALHMQALPPR

SEQ ID NO: 2 - protein, 731 aa, synthetic construct
  REGION 1..731: note = SYNTHETIC
MLLVTSLLLCELPHPAFLLIPEVQLVQSGAEVKKPGSSVKVSCKASGGTFSSYAISWVRQAPGQGLEWMGGIIPIFGTANYAQKFQGRVTITADKSTSTAYMELSSLRSEDTAVYYCATFALFGFREQAFDIWGQGTTVTVSSGGGGSGGGGSGGGGSDIQMTQSPSSLSASVGDRVTITCRASQSISSYLNWYQQKPGKAPKLLIYAASSLQSGVPSRFSGSGSGTDFTLTISSLQPEDLATYYCQQSYSTPFTFGPGTKVDIKSGLEDPAEPKSPDKTHTCPPCPAPELLGGPSVFLFPPKPKDTLMISRTPEVTCVVVDVSHEDPEVKFNWYVDGVEVHNAKTKPREEQYNSTYRVVSVLTVLHQDWLNGKEYKCKVSNKALPAPIEKTISKAKGQPREPQVYTLPPSRDELTKNQVSLTCLVKGFYPSDIAVEWESNGQPENNYKTTPPVLDSDGSFFLYSKLTVDKSRWQQGNVFSCSVMHEALHNHYTQKSLSLSPGKKDPKTTTPAPRPPTPAPTIASQPLSLRPEACRPAAGGAVHTRGLDFACDIYIWAPLAGTCGVLLLSLVITLYCKRGRKKLLYIFKQPFMRPVQTTQEEDGCSCRFPEEEEGGCELRVKFSRSADAPAYKQGQNQLYNELNLGRREEYDVLDKRRGRDPEMGGKPRRKNPQEGLYNELQKDKMAEAYSEIGMKGERRRGKGHDGLYQGLSTATKDTYDALHMQALPPR

SEQ ID NO: 3 - skipped

SEQ ID NO: 4 - protein, 20 aa, synthetic construct
  REGION 1..20: note = SYNTHETIC
LLVTSLLLCELPHPAFLLIP

SEQ ID NO: 5 - protein, 25 aa, synthetic construct
  REGION 1..25: note = SYNTHETIC
EVQLVQSGAEVKKPGSSVKVSCKAS

SEQ ID NO: 6 - protein, 10 aa, synthetic construct
  REGION 1..10: note = SYNTHETIC
GGTFSSYAIS

SEQ ID NO: 7 - protein, 14 aa, synthetic construct
  REGION 1..14: note = SYNTHETIC
WVRQAPGQGLEWMG

SEQ ID NO: 8 - protein, 17 aa, synthetic construct
  REGION 1..17: note = SYNTHETIC
GIIPIFGTANYAQKFQG

SEQ ID NO: 9 - protein, 32 aa, synthetic construct
  REGION 1..32: note = SYNTHETIC
RVTITADKSTSTAYMELSSLRSEDTAVYYCAT

SEQ ID NO: 10 - protein, 13 aa, synthetic construct
  REGION 1..13: note = SYNTHETIC
FALFGFREQAFDI

SEQ ID NO: 11 - protein, 11 aa, synthetic construct
  REGION 1..11: note = SYNTHETIC
WGQGTTVTVSS

SEQ ID NO: 12 - protein, 15 aa, synthetic construct
  REGION 1..15: note = SYNTHETIC
GGGGSGGGGSGGGGS

SEQ ID NO: 13 - protein, 23 aa, synthetic construct
  REGION 1..23: note = SYNTHETIC
DIQMTQSPSSLSASVGDRVTITC

SEQ ID NO: 14 - protein, 11 aa, synthetic construct
  REGION 1..11: note = SYNTHETIC
RASQSISSYLN

SEQ ID NO: 15 - protein, 15 aa, synthetic construct
  REGION 1..15: note = SYNTHETIC
WYQQKPGKAPKLLIY

SEQ ID NO: 16 - protein, 7 aa, synthetic construct
  REGION 1..7: note = SYNTHETIC
AASSLQS

SEQ ID NO: 17 - protein, 32 aa, synthetic construct
  REGION 1..32: note = SYNTHETIC
GVPSRFSGSGSGTDFTLTISSLQPEDLATYYC

SEQ ID NO: 18 - protein, 9 aa, synthetic construct
  REGION 1..9: note = SYNTHETIC
QQSYSTPFT

SEQ ID NO: 19 - protein, 10 aa, synthetic construct
  REGION 1..10: note = SYNTHETIC
FGPGTKVDIK

SEQ ID NO: 20 - skipped

SEQ ID NO: 21 - protein, 4 aa, synthetic construct
  REGION 1..4: note = SYNTHETIC
LEDP

SEQ ID NO: 22 - protein, 126 aa, synthetic construct
  REGION 1..126: note = SYNTHETIC
AEPKSPDKTHTCPPCPAPELLGGPSVFLFPPKPKDTLMISRTPEVTCVVVDVSHEDPEVKFNWYVDGVEVHNAKTKPREEQYNSTYRVVSVLTVLHQDWLNGKEYKCKVSNKALPAPIEKTISKAK

SEQ ID NO: 23 - protein, 107 aa, synthetic construct
  REGION 1..107: note = SYNTHETIC
GQPREPQVYTLPPSRDELTKNQVSLTCLVKGFYPSDIAVEWESNGQPENNYKTTPPVLDSDGSFFLYSKLTVDKSRWQQGNVFSCSVMHEALHNHYTQKSLSLSPGK

SEQ ID NO: 24 - protein, 4 aa, synthetic construct
  REGION 1..4: note = SYNTHETIC
KDPK

SEQ ID NO: 25 - protein, 45 aa, synthetic construct
  REGION 1..45: note = SYNTHETIC
TTTPAPRPPTPAPTIASQPLSLRPEACRPAAGGAVHTRGLDFACD

SEQ ID NO: 26 - protein, 24 aa, synthetic construct
  REGION 1..24: note = SYNTHETIC
IYIWAPLAGTCGVLLLSLVITLYC

SEQ ID NO: 27 - protein, 42 aa, synthetic construct
  REGION 1..42: note = SYNTHETIC
KRGRKKLLYIFKQPFMRPVQTTQEEDGCSCRFPEEEEGGCEL

SEQ ID NO: 28 - protein, 112 aa, synthetic construct
  REGION 1..112: note = SYNTHETIC
RVKFSRSADAPAYKQGQNQLYNELNLGRREEYDVLDKRRGRDPEMGGKPRRKNPQEGLYNELQKDKMAEAYSEIGMKGERRRGKGHDGLYQGLSTATKDTYDALHMQALPPR

SEQ ID NO: 29 - protein, 469 aa, synthetic construct
  REGION 1..469: note = SYNTHETIC
EVQLVQSGAEVKKPGSSVKVSCKASGGTFSSYAISWVRQAPGQGLEWMGGIIPIFGTANYAQKFQGRVTITADKSTSTAYMELSSLRSEDTAVYYCATFALFGFREQAFDIWGQGTTVTVSSGGGGSGGGGSGGGGSDIQMTQSPSSLSASVGDRVTITCRASQSISSYLNWYQQKPGKAPKLLIYAASSLQSGVPSRFSGSGSGTDFTLTISSLQPEDLATYYCQQSYSTPFTFGPGTKVDIKSGTTTPAPRPPTPAPTIASQPLSLRPEACRPAAGGAVHTRGLDFACDIYIWAPLAGTCGVLLLSLVITLYCKRGRKKLLYIFKQPFMRPVQTTQEEDGCSCRFPEEEEGGCELRVKFSRSADAPAYKQGQNQLYNELNLGRREEYDVLDKRRGRDPEMGGKPRRKNPQEGLYNELQKDKMAEAYSEIGMKGERRRGKGHDGLYQGLSTATKDTYDALHMQALPPR

SEQ ID NO: 30 - protein, 710 aa, synthetic construct
  REGION 1..710: note = SYNTHETIC
EVQLVQSGAEVKKPGSSVKVSCKASGGTFSSYAISWVRQAPGQGLEWMGGIIPIFGTANYAQKFQGRVTITADKSTSTAYMELSSLRSEDTAVYYCATFALFGFREQAFDIWGQGTTVTVSSGGGGSGGGGSGGGGSDIQMTQSPSSLSASVGDRVTITCRASQSISSYLNWYQQKPGKAPKLLIYAASSLQSGVPSRFSGSGSGTDFTLTISSLQPEDLATYYCQQSYSTPFTFGPGTKVDIKSGLEDPAEPKSPDKTHTCPPCPAPELLGGPSVFLFPPKPKDTLMISRTPEVTCVVVDVSHEDPEVKFNWYVDGVEVHNAKTKPREEQYNSTYRVVSVLTVLHQDWLNGKEYKCKVSNKALPAPIEKTISKAKGQPREPQVYTLPPSRDELTKNQVSLTCLVKGFYPSDIAVEWESNGQPENNYKTTPPVLDSDGSFFLYSKLTVDKSRWQQGNVFSCSVMHEALHNHYTQKSLSLSPGKKDPKTTTPAPRPPTPAPTIASQPLSLRPEACRPAAGGAVHTRGLDFACDIYIWAPLAGTCGVLLLSLVITLYCKRGRKKLLYIFKQPFMRPVQTTQEEDGCSCRFPEEEEGGCELRVKFSRSADAPAYKQGQNQLYNELNLGRREEYDVLDKRRGRDPEMGGKPRRKNPQEGLYNELQKDKMAEAYSEIGMKGERRRGKGHDGLYQGLSTATKDTYDALHMQALPPR